European Patent Specification EP 4 031 108 B1, published April 2, 2025. Title: Extrudierte Depotform mit kontrollierter Wirkstofffreisetzung. Applicant: AMW GmbH. The sequence listing filed with the application follows.

SEQUENCE LISTING (1 sequence)

SEQ ID NO: 1 - protein, 8 aa, synthetic organisms
  Polypeptid
FCFWKTCT